European Patent Application EP 4 549 431 A1, published May 7, 2025. Title: Compound functioning as smarca2/4 inhibitor and use thereof. Applicant: GAN & LEE PHARMACEUTICALS CO., LTD. Application EP 23 830 537.9, filed June 30, 2023. The sequence listing filed with the application follows.

SEQUENCE LISTING (2 sequences)

SEQ ID NO: 1 - protein, 110 aa, synthetic construct
SPNPPKLTKQMNAIIDTVRNYKDSSGRQLSEVFIQLPSRKELPEYYELIRKPVDFKKIKERIRNHKYRSLGDLEKDVMLLCHNAQTFNLEGSQIYEDSIVLQSVFKSARQ

SEQ ID NO: 2 - protein, 128 aa, synthetic construct
AEKLSPNPPNLTKKMKKIVDAVIKYKDSSSGRQLSEVFIQLPSRKELPEYYELIRKPVDFKKIKERIRNHKYRSLNDLEKDVMLLCQNAQTFNLEGSLIYEDSIVLQSVFTSVRQKIEKEDDSEGEES